European Patent Specification EP 3 725 799 B1, published November 5, 2025. Title: PD-L1 binding peptide and use thereof. Applicant: KYUNGPOOK NATIONAL UNIVERSITY INDUSTRY-ACADEMIC COOPERATION FOUNDATION. The sequence listing filed with the application follows.

SEQUENCE LISTING (2 sequences)

SEQ ID NO: 1 - protein, 9 aa, Artificial Sequence
  synthetic peptide
CLQKTPKQC

SEQ ID NO: 2 - protein, 7 aa, Artificial Sequence
  synthetic peptide
CVRARTR